European Patent Application EP 4 458 977 A1, published November 6, 2024. Title: Self-assembling peptide amphiphiles as retroviral transduction enhancers. Applicant: Max-Planck-Gesellschaft zur Förderung der Wissenschaften e.V. The sequence listing filed with the application follows.

SEQUENCE LISTING (101 sequences)

SEQ ID NO: 1 - protein, 9 aa, synthetic construct
  source 1..9: note = Peptide P1
  MOD_RES 9: note = AMIDATION; note = lysine amide
VVVAAAKKK

SEQ ID NO: 2 - protein, 9 aa, synthetic construct
  source 1..9: note = Peptide P3
  MOD_RES 9: note = AMIDATION; note = glutamic acid amide
VVVAAAEEE

SEQ ID NO: 3 - protein, 7 aa, synthetic construct
  source 1..7: note = Peptide P2
  MOD_RES 7: note = AMIDATION; note = cysteine amide
FQFKFKC

SEQ ID NO: 4 - protein, 9 aa, synthetic construct
  source 1..9: note = Peptide Amphiphile PA1
  MOD_RES 9: note = lysine amide; note = AMIDATION
  LIPID 1: note = N-palmitoyl valine; note = PALMITATE
VVVAAAKKK

SEQ ID NO: 5 - protein, 9 aa, synthetic construct
  source 1..9: note = Peptide Amphiphile PA3
  MOD_RES 9: note = glutamic acide amide; note = AMIDATION
  LIPID 1: note = PALMITATE; note = N-palmitoyl valine
VVVAAAEEE

SEQ ID NO: 6 - protein, 7 aa, synthetic construct
  source 1..7: note = Reverse Peptide P2
  MOD_RES 7: note = AMIDATION; note = phenylalanine amide
CKFKFQF

SEQ ID NO: 7 - protein, 7 aa, synthetic construct
  source 1..7: note = Peptide Amphiphile PA2
  MOD_RES 7: note = AMIDATION; note = phenylalanine amide
  LIPID 1: note = N-palmitoyl cysteine; note = PALMITATE
CKFKFQF

SEQ ID NO: 8 - protein, 7 aa, synthetic construct
  source 1..7: note = Peptide Amphiphile Reverse PA2
  MOD_RES 7: note = cysteine amide; note = AMIDATION
  LIPID 1: note = N-palmitoyl phenylalanine; note = PALMITATE
FQFKFKC

SEQ ID NO: 9 - protein, 12 aa, synthetic construct
  source 1..12: note = EF-C
QCKIKQIINMWQ

SEQ ID NO: 10 - protein, 10 aa, synthetic construct
  source 1..10: note = Peptide Amphiphile Pat1
  MOD_RES 10: note = lysine amide; note = AMIDATION
  LIPID 1: note = O-palmitoyl serine; note = PALMITATE
SVVVAAAKKK

SEQ ID NO: 11 - protein, 10 aa, synthetic construct
  source 1..10: note = Peptide Amphiphile Pat2
  MOD_RES 10: note = lysine amide; note = AMIDATION
  MOD_RES 1: note = HEXADECANYLDISULFID; note = hexadecanyl-S-S-cysteine
CVVVAAAKKK

SEQ ID NO: 12 - protein, 10 aa, synthetic construct
  source 1..10: note = Peptide Amphiphile Pat3
  MOD_RES 10: note = lysine amide; note = AMIDATION
  LIPID 1: note = PALMITATE; note = S-palmitoyl-cysteine
CVVVAAAKKK

SEQ ID NO: 13 - protein, 5 aa, synthetic construct
  source 1..5: note = Second Peptide Part Pat19
LNGGV

SEQ ID NO: 14 - protein, 9 aa, synthetic construct
  source 1..9: note = Peptide Amphiphile Pat10
  MOD_RES 9: note = lysine amide; note = AMIDATION
  LIPID 1: note = N-Eicosapentaenoic acid modified valine; note = Eicosapentaenoate
VVVAAAKKK

SEQ ID NO: 15 - protein, 9 aa, synthetic construct
  source 1..9: note = Peptide Amphiphile Pat7
  MOD_RES 9: note = AMIDATION; note = lysine amide
  LIPID 1: note = N-lauroyl valine; note = LAURATE
VVVAAAKKK

SEQ ID NO: 16 - protein, 9 aa, synthetic construct
  source 1..9: note = Peptide Amphiphile Pat8
  MOD_RES 9: note = lysine amide; note = AMIDATION
  LIPID 1: note = N-perlagonoyl valine; note = PERLAGONATE
VVVAAAKKK

SEQ ID NO: 17 - protein, 9 aa, synthetic construct
  source 1..9: note = Peptide Amphiphile Pat12
  MOD_RES 9: note = AMIDATION; note = lysine amide
  MOD_RES 1: note = N-Fluorenylmethoxycarbonyl valine; note = Fluorenylmethoxycarbonyl
VVVAAAKKK

SEQ ID NO: 18 - protein, 9 aa, synthetic construct
  source 1..9: note = Peptide Amphiphile Pat13
  MOD_RES 9: note = AMIDATION; note = lysine amide
  MOD_RES 1: note = 2-naphthylmethyl; note = N-2-naphthylmethyl valine
VVVAAAKKK

SEQ ID NO: 19 - protein, 9 aa, synthetic construct
  source 1..9: note = Peptide Amphiphile Pat9
  MOD_RES 9: note = AMIDATION; note = lysine amide
  LIPID 1: note = N-alpha-linolenic acid modified valine; note = ALPHA-LINEOATE
VVVAAAKKK

SEQ ID NO: 20 - protein, 7 aa, synthetic construct
  source 1..7: note = Peptide Amphiphile Pat19
  MOD_RES 7: note = lysine amide; note = AMIDATION
  LIPID 1: note = PALMITATE; note = N-palmitoyl leucine
LNGGVKK

SEQ ID NO: 21 - protein, 7 aa, synthetic construct
  source 1..7: note = Peptide Pat38
  MOD_RES 7: note = lysine amide; note = AMIDATION
LNGGVKK

SEQ ID NO: 22 - protein, 7 aa, synthetic construct
  source 1..7: note = Peptide Amphiphile Pat20
  MOD_RES 7: note = AMIDATION; note = lysine amide
  LIPID 1: note = PALMITATE; note = N-palmitoyl alanine
ALAAGKK

SEQ ID NO: 23 - protein, 7 aa, synthetic construct
  source 1..7: note = Peptide Pat39
  MOD_RES 7: note = lysine amide; note = AMIDATION
ALAAGKK

SEQ ID NO: 24 - protein, 6 aa, synthetic construct
  source 1..6: note = Peptide Amphiphile Pat31
  MOD_RES 6: note = AMIDATION; note = lysine amide
  LIPID 1: note = PALMITATE; note = N-palmitoyl alanine
AKAVGK

SEQ ID NO: 25 - protein, 6 aa, synthetic construct
  source 1..6: note = Peptide Pat50
  MOD_RES 6: note = lysine amide; note = AMIDATION
AKAVGK

SEQ ID NO: 26 - protein, 6 aa, synthetic construct
  source 1..6: note = Peptide Amphiphile Pat15
  MOD_RES 6: note = AMIDATION; note = lysine amide
  LIPID 1: note = N-palmitoyl isoleucine; note = PALMITATE
IIQKIK

SEQ ID NO: 27 - protein, 6 aa, synthetic construct
  source 1..6: note = Peptide Pat34
  MOD_RES 6: note = lysine amide; note = AMIDATION
IIQKIK

SEQ ID NO: 28 - protein, 6 aa, synthetic construct
  source 1..6: note = Peptide Amphiphile Pat18
  MOD_RES 6: note = AMIDATION; note = lysine amide
  LIPID 1: note = N-palmitoyl alanine; note = PALMITATE
AGGRVK

SEQ ID NO: 29 - protein, 6 aa, synthetic construct
  source 1..6: note = Peptide Pat37
  MOD_RES 6: note = AMIDATION; note = lysine amide
AGGRVK

SEQ ID NO: 30 - protein, 5 aa, synthetic construct
  source 1..5: note = Peptide Amphiphile Pat23
  MOD_RES 5: note = lysine amide; note = AMIDATION
  LIPID 1: note = PALMITATE; note = N-palmitoyl leucine
LLLKK

SEQ ID NO: 31 - protein, 5 aa, synthetic construct
  source 1..5: note = Peptide Pat42
  MOD_RES 5: note = AMIDATION; note = lysine amide
LLLKK

SEQ ID NO: 32 - protein, 9 aa, synthetic construct
  source 1..9: note = Peptide Amphiphile Pat14
  SITE 1: note = D-valine
  SITE 2: note = D-valine
  SITE 3: note = D-valine
  SITE 4: note = D-alanine
  SITE 5: note = D-alanine
  SITE 6: note = D-alanine
  SITE 7: note = D-lysine
  SITE 8: note = D-lysine
  MOD_RES 9: note = AMIDATION; note = D-lysine amide
  SITE 9: note = D-lysine
  LIPID 1: note = PALMITATE; note = N-palmitoyl D-valine
VVVAAAKKK

SEQ ID NO: 33 - protein, 9 aa, synthetic construct
  source 1..9: note = Peptide Pat33
  SITE 1: note = D-valine
  SITE 2: note = D-valine
  SITE 3: note = D-valine
  SITE 4: note = D-alanine
  SITE 5: note = D-alanine
  SITE 6: note = D-alanine
  SITE 7: note = D-lysine
  SITE 8: note = D-lysine
  SITE 9: note = D-lysine
  MOD_RES 9: note = D-lysine amide; note = AMIDATION
VVVAAAKKK

SEQ ID NO: 34 - protein, 6 aa, synthetic construct
  source 1..6: note = Peptide Amphiphile Pat16
  MOD_RES 6: note = lysine amide; note = AMIDATION
  LIPID 1: note = N-palmitoyl alanine; note = PALMITATE
AQAKAK

SEQ ID NO: 35 - protein, 6 aa, synthetic construct
  source 1..6: note = Peptide Pat35
  MOD_RES 6: note = lysine amide; note = AMIDATION
AQAKAK

SEQ ID NO: 36 - protein, 6 aa, synthetic construct
  source 1..6: note = Peptide Amphiphile Pat17
  MOD_RES 6: note = AMIDATION; note = lysine amide
  LIPID 1: note = N-palmitoyl phenylalanine; note = PALMITATE
WEALKK

SEQ ID NO: 37 - protein, 6 aa, synthetic construct
  source 1..6: note = Peptide Pat36
  MOD_RES 6: note = AMIDATION; note = lysine amide
WEALKK

SEQ ID NO: 38 - protein, 6 aa, synthetic construct
  source 1..6: note = Peptide Amphiphile Pat21
  MOD_RES 6: note = AMIDATION; note = lysine amide
  LIPID 1: note = PALMITATE; note = N-palmitoyl alanine
AVAKKK

SEQ ID NO: 39 - protein, 6 aa, synthetic construct
  source 1..6: note = Peptide Pat40
  MOD_RES 6: note = AMIDATION; note = lysine amide
AVAKKK

SEQ ID NO: 40 - protein, 6 aa, synthetic construct
  source 1..6: note = Peptide Amphiphile Pat22
  MOD_RES 6: note = AMIDATION; note = arginine amide
  LIPID 1: note = PALMITATE; note = N-palmitoyl arginine
RRWQWR

SEQ ID NO: 41 - protein, 6 aa, synthetic construct
  source 1..6: note = Peptide Pat41
  MOD_RES 6: note = AMIDATION; note = arginine amide
RRWQWR

SEQ ID NO: 42 - protein, 7 aa, synthetic construct
  source 1..7: note = Peptide Amphiphile Pat24
  LIPID 1: note = N-palmitoyl valine; note = PALMITATE
  MOD_RES 7: note = AMIDATION; note = histidine amide
VVAAHHH

SEQ ID NO: 43 - protein, 7 aa, synthetic construct
  source 1..7: note = Peptide Pat43
  MOD_RES 7: note = histidine amide; note = AMIDATION
VVAAHHH

SEQ ID NO: 44 - protein, 8 aa, synthetic construct
  source 1..8: note = Peptide Amphiphile Pat25
  MOD_RES 8: note = lysine amide; note = AMIDATION
  LIPID 1: note = N-palmitoyl lysine; note = PALMITATE
KGVPGVGK

SEQ ID NO: 45 - protein, 8 aa, synthetic construct
  source 1..8: note = Peptide Pat44
  MOD_RES 8: note = AMIDATION; note = lysine amide
KGVPGVGK

SEQ ID NO: 46 - protein, 16 aa, synthetic construct
  source 1..16: note = Peptide Amphiphile Pat26
  MOD_RES 16: note = AMIDATION; note = valine amide
  LIPID 1: note = PALMITATE; note = N-palmitoyl lysine
KYIHQNYTKALAGKLV

SEQ ID NO: 47 - protein, 16 aa, synthetic construct
  source 1..16: note = Peptide Pat45
  MOD_RES 16: note = AMIDATION; note = valine amide
KYIHQNYTKALAGKLV

SEQ ID NO: 48 - protein, 11 aa, synthetic construct
  source 1..11: note = Peptide Amphiphile Pat27
  MOD_RES 11: note = lysine amide; note = AMIDATION
  LIPID 1: note = PALMITATE; note = N-palmitoyl asparagine
NFYLQVNKINK

SEQ ID NO: 49 - protein, 11 aa, synthetic construct
  source 1..11: note = Peptide Pat46
  MOD_RES 11: note = lysine amide; note = AMIDATION
NFYLQVNKINK

SEQ ID NO: 50 - protein, 8 aa, synthetic construct
  source 1..8: note = Peptide Amphiphile Pat28
  MOD_RES 8: note = AMIDATION; note = lysine amide
  LIPID 1: note = PALMITATE; note = N-palmitoyl glycine
GGGSSKKK

SEQ ID NO: 51 - protein, 8 aa, synthetic construct
  source 1..8: note = Peptide Pat47
  MOD_RES 8: note = AMIDATION; note = lysine amide
GGGSSKKK

SEQ ID NO: 52 - protein, 18 aa, synthetic construct
  source 1..18: note = Peptide Amphiphile Pat29
  MOD_RES 18: note = AMIDATION; note = tyrosine amide
  LIPID 1: note = PALMITATE; note = N-palmitoyl arginine
RYYASLRHYLNLVTRQRY

SEQ ID NO: 53 - protein, 18 aa, synthetic construct
  source 1..18: note = Peptide Pat48
  MOD_RES 18: note = AMIDATION; note = tyrosine amide
RYYASLRHYLNLVTRQRY

SEQ ID NO: 54 - protein, 6 aa, synthetic construct
  source 1..6: note = Peptide Amphiphile Pat30
  MOD_RES 6: note = lysine amide; note = AMIDATION
  LIPID 1: note = PALMITATE; note = N-palmitoyl glycine
GKVGSK

SEQ ID NO: 55 - protein, 6 aa, synthetic construct
  source 1..6: note = Peptide Pat49
  MOD_RES 6: note = lysine amide; note = AMIDATION
GKVGSK

SEQ ID NO: 56 - protein, 6 aa, synthetic construct
  source 1..6: note = Peptide Amphiphile Pat32
  MOD_RES 6: note = AMIDATION; note = lysine amide
  LIPID 1: note = PALMITATE; note = N-palmitoyl lysine
KIISFK

SEQ ID NO: 57 - protein, 6 aa, synthetic construct
  source 1..6: note = Peptide Pat51
  MOD_RES 6: note = AMIDATION; note = lysine amide
KIISFK

SEQ ID NO: 58 - protein, 7 aa, synthetic construct
  source 1..7: note = Peptide Amphiphile Pat52star
  MOD_RES 7: note = lysine amide; note = AMIDATION
  LIPID 1: note = N-palmitoyl alanine; note = PALMITATE
AAVVHHK

SEQ ID NO: 59 - protein, 7 aa, synthetic construct
  source 1..7: note = Peptide Pat52
  MOD_RES 7: note = AMIDATION; note = lysine amide
AAVVHHK

SEQ ID NO: 60 - protein, 6 aa, synthetic construct
  source 1..6: note = Peptide Amphiphile Patistar
  MOD_RES 6: note = AMIDATION; note = arginine amide
  LIPID 1: note = PALMITATE; note = N-palmitoyl glycine
GGVVRR

SEQ ID NO: 61 - protein, 6 aa, synthetic construct
  source 1..6: note = Peptide Pati
  MOD_RES 6: note = AMIDATION; note = arginine amide
GGVVRR

SEQ ID NO: 62 - protein, 7 aa, synthetic construct
  source 1..7: note = Peptide Amphiphile Patjstar
  MOD_RES 7: note = AMIDATION; note = arginine amide
  LIPID 1: note = N-palmitoyl alanine; note = PALMITATE
AGAGRRR

SEQ ID NO: 63 - protein, 7 aa, synthetic construct
  source 1..7: note = Peptide Patj
  MOD_RES 7: note = AMIDATION; note = arginine amide
AGAGRRR

SEQ ID NO: 64 - protein, 5 aa, synthetic construct
  source 1..5: note = second peptide part Pat 20
ALAAG

SEQ ID NO: 65 - protein, 5 aa, synthetic construct
  source 1..5: note = second peptide part Pat31
AKAVG

SEQ ID NO: 66 - protein, 7 aa, synthetic construct
CVVVAAA

SEQ ID NO: 67 - protein, 7 aa, synthetic construct
SVVVAAA

SEQ ID NO: 68 - protein, 6 aa, synthetic construct
CLNGGV

SEQ ID NO: 69 - protein, 6 aa, synthetic construct
SLNGGV

SEQ ID NO: 70 - protein, 6 aa, synthetic construct
CALAAG

SEQ ID NO: 71 - protein, 6 aa, synthetic construct
SALAAG

SEQ ID NO: 72 - protein, 6 aa, synthetic construct
CAKAVG

SEQ ID NO: 73 - protein, 6 aa, synthetic construct
SAKAVG

SEQ ID NO: 74 - protein, 6 aa, synthetic construct
VVVAAA

SEQ ID NO: 75 - protein, 9 aa, synthetic construct
VVVAAAKKK

SEQ ID NO: 76 - protein, 10 aa, synthetic construct
CVVVAAAKKK

SEQ ID NO: 77 - protein, 10 aa, synthetic construct
SVVVAAAKKK

SEQ ID NO: 78 - protein, 7 aa, synthetic construct
LNGGVKK

SEQ ID NO: 79 - protein, 7 aa, synthetic construct
ALAAGKK

SEQ ID NO: 80 - protein, 6 aa, synthetic construct
AKAVGK

SEQ ID NO: 81 - protein, 6 aa, synthetic construct
IIQKIK

SEQ ID NO: 82 - protein, 6 aa, synthetic construct
AGGRVK

SEQ ID NO: 83 - protein, 5 aa, synthetic construct
LLLKK

SEQ ID NO: 84 - protein, 6 aa, synthetic construct
AQAKAK

SEQ ID NO: 85 - protein, 6 aa, synthetic construct
WEALKK

SEQ ID NO: 86 - protein, 6 aa, synthetic construct
AVAKKK

SEQ ID NO: 87 - protein, 7 aa, synthetic construct
CKFKFQF

SEQ ID NO: 88 - protein, 6 aa, synthetic construct
RRWQWR

SEQ ID NO: 89 - protein, 7 aa, synthetic construct
VVAAHHH

SEQ ID NO: 90 - protein, 8 aa, synthetic construct
KGVPGVGK

SEQ ID NO: 91 - protein, 16 aa, synthetic construct
KYIHQNYTKALAGKLV

SEQ ID NO: 92 - protein, 11 aa, synthetic construct
NFYLQVNKINK

SEQ ID NO: 93 - protein, 8 aa, synthetic construct
GGGSSKKK

SEQ ID NO: 94 - protein, 18 aa, synthetic construct
RYYASLRHYLNLVTRQRY

SEQ ID NO: 95 - protein, 6 aa, synthetic construct
GKVGSK

SEQ ID NO: 96 - protein, 6 aa, synthetic construct
KIISFK

SEQ ID NO: 97 - protein, 7 aa, synthetic construct
AAVVHHK

SEQ ID NO: 98 - protein, 6 aa, synthetic construct
GGVVRR

SEQ ID NO: 99 - protein, 7 aa, synthetic construct
AGAGRRR

SEQ ID NO: 100 - protein, 9 aa, synthetic construct
VVVAAAEEE

SEQ ID NO: 101 - protein, 7 aa, synthetic construct
FQFKFKC